European Patent Application EP 4 446 429 A1, published October 16, 2024. Title: Double strand nucleic acid Tm raising agent. Applicant: 日東紡績株式会社. The sequence listing filed with the application follows.

SEQUENCE LISTING (4 sequences)

SEQ ID NO: 1 - DNA, 11 bp, Homo sapiens
  misc_feature 1..11: note = oligo DNA derived from Exon 2 of WT KRAS gene sense chain
  source 1..11: mol_type = genomic DNA
ggtggcgtagg

SEQ ID NO: 2 - DNA, 11 bp, Homo sapiens
  misc_feature 1..11: note = oligo DNA derived from Exon 2 of WT KRAS gene antisense chain
  source 1..11: mol_type = genomic DNA
cctacgccacc

SEQ ID NO: 3 - DNA, 11 bp, synthetic construct
  misc_feature 1..11: note = oligo DNA derived from mutant KRAS gene sense chain
  source 1..11: mol_type = other DNA
ggtgacgtagg

SEQ ID NO: 4 - DNA, 11 bp, synthetic construct
  misc_feature 1..11: note = BNA derived from Exon 2 of WT KRAS gene antisense chain
  misc_feature 1..2: note = 2',4'-BNANC(N-H)-cytosine
  misc_feature 3: note = 2',4'-BNANC(N-H)-thymine
  misc_feature 5: note = 2',4'-BNANC(N-H)-cytosine
  misc_feature 7..8: note = 2',4'-BNANC(N-H)-cytosine
  misc_feature 10..11: note = 2',4'-BNANC(N-H)-cytosine
  source 1..11: mol_type = other DNA
cctacgccacc